European Patent Application EP 4 667 058 A2, published December 24, 2025. Title: ANTI-BCMA ANTIBODIES, BISPECIFIC ANTIGEN BINDING MOLECULES THAT BIND BCMA AND CD3, AND USES THEREOF. Applicant: JANSSEN PHARMACEUTICA NV. The sequence listing filed with the application follows.

SEQUENCE LISTING (77 sequences)

SEQ ID NO: 1 - protein, 184 aa, Homo sapiens
MLQMAGQCSQNEYFDSLLHACIPCQLRCSSNTPPLTCQRYCNASVTNSVKGTNAILWTCLGLSLIISLAVFVLMFLLRKINSEPLKDEFKNTGSGLLGMANIDLEKSRTGDEIILPRGLEYTVEECTCEDCIKSKPKVDSDHCFPLPAMEEGATILVTTKTNDYCKSLPAALSATEIEKSISAR

SEQ ID NO: 2 - protein, 185 aa, Mus sp.
MAQQCFHSEYFDSLLHACKPCHLRCSNPPATCQPYCDPSVTSSVKGTYTVLWIFLGLTLVLSLALFTISFLLRKMNPEALKDEPQSPGQLDGSAQLDKADTELTRIRAGDDRIFPRSLEYTVEECTCEDCVKSKPKGDSDHFFPLPAMEEGATILVTTKTGDYGKSSVPTALQSVMGMEKPTHTR

SEQ ID NO: 3 - protein, 183 aa, Macaca fascicularis
MLQMARQCSQNEYFDSLLHDCKPCQLRCSSTPPLTCQRYCNASMTNSVKGMNAILWTCLGLSLIISLAVFVLTFLLRKMSSEPLKDEFKNTGSGLLGMANIDLEKGRTGDEIVLPRGLEYTVEECTCEDCIKNKPKVDSDHCFPLPAMEEGATILVTTKTNDYCNSLSAALSVTEIEKSISAR

SEQ ID NO: 4 - protein, 7 aa, Homo sapiens
SGSYFWG

SEQ ID NO: 5 - protein, 16 aa, Homo sapiens
SIYYSGITYYNPSLKS

SEQ ID NO: 6 - protein, 11 aa, Homo sapiens
HDGAVAGLFDY

SEQ ID NO: 7 - protein, 7 aa, Homo sapiens
SSSYYWG

SEQ ID NO: 8 - protein, 16 aa, Homo sapiens
SIYYSGSTYYNPSLKS

SEQ ID NO: 9 - protein, 11 aa, Homo sapiens
HDAATAGLFDY

SEQ ID NO: 10 - protein, 7 aa, Homo sapiens
SGSYYWG

SEQ ID NO: 11 - protein, 16 aa, Homo sapiens
SIYYSGWTYYNPSLKS

SEQ ID NO: 12 - protein, 11 aa, Homo sapiens
HEGATAGLFDY

SEQ ID NO: 13 - protein, 7 aa, Homo sapiens
SSSYFWG

SEQ ID NO: 14 - protein, 16 aa, Homo sapiens
SIYYSGRTYYNPSLKS

SEQ ID NO: 15 - protein, 11 aa, Homo sapiens
HSGATAGLFDY

SEQ ID NO: 16 - protein, 11 aa, Homo sapiens
HEGAVAGLFDY

SEQ ID NO: 17 - protein, 11 aa, Homo sapiens
HSGAVAGLFDY

SEQ ID NO: 18 - protein, 11 aa, Homo sapiens
HDAAVAGLFDY

SEQ ID NO: 19 - protein, 11 aa, Homo sapiens
HDGATAGLFDY

SEQ ID NO: 20 - protein, 11 aa, Homo sapiens
HQGATAGLFDY

SEQ ID NO: 21 - protein, 11 aa, Homo sapiens
HHGATAGLFDY

SEQ ID NO: 22 - protein, 11 aa, Homo sapiens
HWGATAGLFDY

SEQ ID NO: 23 - protein, 11 aa, Homo sapiens
HYGATAGLFDY

SEQ ID NO: 24 - protein, 11 aa, Homo sapiens
GGNNIGSKSVH

SEQ ID NO: 25 - protein, 7 aa, Homo sapiens
DDSDRPS

SEQ ID NO: 26 - protein, 11 aa, Homo sapiens
QVWDSSSDHVV

SEQ ID NO: 27 - protein, 122 aa, Homo sapiens
QLQLQESGPGLVKPSETLSLTCTVSGGSISSGSYFWGWIRQPPGKGLEWIGSIYYSGITYYNPSLKSRVTISVDTSKNQFSLKLSSVTAADTAVYYCARHDGAVAGLFDYWGQGTLVTVSSA

SEQ ID NO: 28 - protein, 108 aa, Homo sapiens
SYVLTQPPSVSVAPGQTARITCGGNNIGSKSVHWYQQPPGQAPVVVVYDDSDRPSGIPERFSGSNSGNTATLTISRVEAGDEAVYYCQVWDSSSDHVVFGGGTKLTVL

SEQ ID NO: 29 - protein, 122 aa, Homo sapiens
QLQLQESGPGLVKPSETLSLTCTVSGGSISSGSYYWGWIRQPPGKGLEWIGSIYYSGITYYNPSLKSRVTISVDTSKNQFSLKLSSVTAADTAVYYCARHDAATAGLFDYWGQGTLVTVSSA

SEQ ID NO: 30 - protein, 108 aa, Homo sapiens
SYVLTQPPSVSVAPGQTARITCGGNNIGSKSVHWYQQKPGQAPVLVVYDDSDRPSGIPERFSGSNSGNTATLTISRVEAGDEADYYCQVWDSSSDHVVFGGGTKLTVL

SEQ ID NO: 31 - protein, 122 aa, Homo sapiens
QLQLQESGPGLVKPSETLSLTCTVSGGSISSGSYYWGWIRQPPGKGLEWIGSIYYSGITYYNPSLKSRVTISVDTSKNQFSLKLSSVTAADTAVYYCARHEGATAGLFDYWGQGTLVTVSSA

SEQ ID NO: 32 - protein, 122 aa, Homo sapiens
QLQLQESGPGLVKPSETLSLTCTVSGGSISSGSYYWGWIRQPPGKGLEWIGSIYYSGITYYNPSLKSRVTISVDTSKNQFSLKLSSVTAADTAVYYCARHSGATAGLFDYWGQGTLVTVSSA

SEQ ID NO: 33 - protein, 122 aa, Homo sapiens
QLQLQESGPGLVKPSETLSLTCTVSGGSISSSSYYWGWIRQPPGKGLEWIGSIYYSGSTYYNPSLKSRVTISVDTSKNQFSLKLSSVTAADTAVYYCARHDGAVAGLFDYWGQGTLVTVSSA

SEQ ID NO: 34 - protein, 122 aa, Homo sapiens
QLQLQESGPGLVKPSETLSLTCTVSGGSISSSSYFWGWIRQPPGKGLEWIGSIYYSGITYYNPSLKSRVTISVDTSKNQFSLKLSSVTAADTAVYYCARHDGAVAGLFDYWGQGTLVTVSSA

SEQ ID NO: 35 - protein, 122 aa, Homo sapiens
QLQLQESGPGLVKPSETLSLTCTVSGGSISSGSYYWGWIRQPPGKGLEWIGSIYYSGITYYNPSLKSRVTISVDTSKNQFSLKLSSVTAADTAVYYCARHDGAVAGLFDYWGQGTLVTVSSA

SEQ ID NO: 36 - protein, 122 aa, Homo sapiens
QLQLQESGPGLVKPSETLSLTCTVSGGSISSGSYFWGWIRQPPGKGLEWIGSIYYSGITYYNPSLKSRVTISVDTSKNQFSLKLSSVTAADTAVYYCARHEGAVAGLFDYWGQGTLVTVSSA

SEQ ID NO: 37 - protein, 122 aa, Homo sapiens
QLQLQESGPGLVKPSETLSLTCTVSGGSISSGSYFWGWIRQPPGKGLEWIGSIYYSGITYYNPSLKSRVTISVDTSKNQFSLKLSSVTAADTAVYYCARHSGAVAGLFDYWGQGTLVTVSSA

SEQ ID NO: 38 - protein, 122 aa, Homo sapiens
QLQLQESGPGLVKPSETLSLTCTVSGGSISSGSYFWGWIRQPPGKGLEWIGSIYYSGITYYNPSLKSRVTISVDTSKNQFSLKLSSVTAADTAVYYCARHDAAVAGLFDYWGQGTLVTVSSA

SEQ ID NO: 39 - protein, 122 aa, Homo sapiens
QLQLQESGPGLVKPSETLSLTCTVSGGSISSGSYFWGWIRQPPGKGLEWIGSIYYSGITYYNPSLKSRVTISVDTSKNQFSLKLSSVTAADTAVYYCARHDGATAGLFDYWGQGTLVTVSSA

SEQ ID NO: 40 - protein, 122 aa, Homo sapiens
QLQLQESGPGLVKPSETLSLTCTVSGGSISSGSYFWGWIRQPPGKGLEWIGSIYYSGSTYYNPSLKSRVTISVDTSKNQFSLKLSSVTAADTAVYYCARHDGAVAGLFDYWGQGTLVTVSSA

SEQ ID NO: 41 - protein, 122 aa, Homo sapiens
QLQLQESGPGLVKPSETLSLTCTVSGGSISSGSYYWGWIRQPPGKGLEWIGSIYYSGSTYYNPSLKSRVTISVDTSKNQFSLKLSSVTAADTAVYYCARHDAAVAGLFDYWGQGTLVTVSSA

SEQ ID NO: 42 - protein, 122 aa, Homo sapiens
QLQLQESGPGLVKPSETLSLTCTVSGGSISSGSYYWGWIRQPPGKGLEWIGSIYYSGSTYYNPSLKSRVTISVDTSKNQFSLKLSSVTAADTAVYYCARHEGAVAGLFDYWGQGTLVTVSSA

SEQ ID NO: 43 - protein, 122 aa, Homo sapiens
QLQLQESGPGLVKPSETLSLTCTVSGGSISSSSYFWGWIRQPPGKGLEWIGSIYYSGRTYYNPSLKSRVTISVDTSKNQFSLKLSSVTAADTAVYYCARHDGATAGLFDYWGQGTLVTVSSA

SEQ ID NO: 44 - protein, 122 aa, Homo sapiens
QLQLQESGPGLVKPSETLSLTCTVSGGSISSSSYFWGWIRQPPGKGLEWIGSIYYSGWTYYNPSLKSRVTISVDTSKNQFSLKLSSVTAADTAVYYCARHDGATAGLFDYWGQGTLVTVSSA

SEQ ID NO: 45 - protein, 122 aa, Homo sapiens
QLQLQESGPGLVKPSETLSLTCTVSGGSISSSSYFWGWIRQPPGKGLEWIGSIYYSGITYYNPSLKSRVTISVDTSKNQFSLKLSSVTAADTAVYYCARHQGATAGLFDYWGQGTLVTVSSA

SEQ ID NO: 46 - protein, 122 aa, Homo sapiens
QLQLQESGPGLVKPSETLSLTCTVSGGSISSSSYFWGWIRQPPGKGLEWIGSIYYSGITYYNPSLKSRVTISVDTSKNQFSLKLSSVTAADTAVYYCARHHGATAGLFDYWGQGTLVTVSSA

SEQ ID NO: 47 - protein, 122 aa, Homo sapiens
QLQLQESGPGLVKPSETLSLTCTVSGGSISSSSYFWGWIRQPPGKGLEWIGSIYYSGITYYNPSLKSRVTISVDTSKNQFSLKLSSVTAADTAVYYCARHWGATAGLFDYWGQGTLVTVSSA

SEQ ID NO: 48 - protein, 122 aa, Homo sapiens
QLQLQESGPGLVKPSETLSLTCTVSGGSISSSSYFWGWIRQPPGKGLEWIGSIYYSGITYYNPSLKSRVTISVDTSKNQFSLKLSSVTAADTAVYYCARHYGATAGLFDYWGQGTLVTVSSA

SEQ ID NO: 49 - protein, 122 aa, Homo sapiens
QLQLQESGPGLVKPSETLSLTCTVSGGSISSSSYFWGWIRQPPGKGLEWIGSIYYSGRTYYNPSLKSRVTISVDTSKNQFSLKLSSVTAADTAVYYCARHQGATAGLFDYWGQGTLVTVSSA

SEQ ID NO: 50 - protein, 122 aa, Homo sapiens
QLQLQESGPGLVKPSETLSLTCTVSGGSISSSSYFWGWIRQPPGKGLEWIGSIYYSGRTYYNPSLKSRVTISVDTSKNQFSLKLSSVTAADTAVYYCARHHGATAGLFDYWGQGTLVTVSSA

SEQ ID NO: 51 - protein, 122 aa, Homo sapiens
QLQLQESGPGLVKPSETLSLTCTVSGGSISSSSYFWGWIRQPPGKGLEWIGSIYYSGRTYYNPSLKSRVTISVDTSKNQFSLKLSSVTAADTAVYYCARHYGATAGLFDYWGQGTLVTVSSA

SEQ ID NO: 52 - protein, 122 aa, Homo sapiens
QLQLQESGPGLVKPSETLSLTCTVSGGSISSSSYFWGWIRQPPGKGLEWIGSIYYSGWTYYNPSLKSRVTISVDTSKNQFSLKLSSVTAADTAVYYCARHQGATAGLFDYWGQGTLVTVSSA

SEQ ID NO: 53 - protein, 122 aa, Homo sapiens
QLQLQESGPGLVKPSETLSLTCTVSGGSISSSSYFWGWIRQPPGKGLEWIGSIYYSGWTYYNPSLKSRVTISVDTSKNQFSLKLSSVTAADTAVYYCARHHGATAGLFDYWGQGTLVTVSSA

SEQ ID NO: 54 - protein, 122 aa, Homo sapiens
QLQLQESGPGLVKPSETLSLTCTVSGGSISSSSYFWGWIRQPPGKGLEWIGSIYYSGWTYYNPSLKSRVTISVDTSKNQFSLKLSSVTAADTAVYYCARHYGATAGLFDYWGQGTLVTVSSA

SEQ ID NO: 55 - protein, 452 aa, Homo sapiens
EVQLVESGGGLVQPGGSLRLSCAASGFTFNTYAMNWVRQAPGKGLEWVARIRSKYNNYATYYAASVKGRFTISRDDSKNSLYLQMNSLKTEDTAVYYCARHGNFGNSYVSWFAYWGQGTLVTVSSASTKGPSVFPLAPCSRSTSESTAALGCLVKDYFPEPVTVSWNSGALTSGVHTFPAVLQSSGLYSLSSVVTVPSSSLGTKTYTCNVDHKPSNTKVDKRVESKYGPPCPPCPAPEAAGGPSVFLFPPKPKDTLMISRTPEVTCVVVDVSQEDPEVQFNWYVDGVEVHNAKTKPREEQFNSTYRVVSVLTVLHQDWLNGKEYKCKVSNKGLPSSIEKTISKAKGQPREPQVYTLPPSQEEMTKNQVSLTCLVKGFYPSDIAVEWESNGQPENNYKTTPPVLDSDGSFLLYSKLTVDKSRWQEGNVFSCSVMHEALHNHYTQKSLSLSLGK

SEQ ID NO: 56 - protein, 215 aa, Homo sapiens
QTVVTQEPSLTVSPGGTVTLTCRSSTGAVTTSNYANWVQQKPGQAPRGLIGGTNKRAPGTPARFSGSLLGGKAALTLSGVQPEDEAEYYCALWYSNLWVFGGGTKLTVLGQPKAAPSVTLFPPSSEELQANKATLVCLISDFYPGAVTVAWKADSSPVKAGVETTTPSKQSNNKYAASSYLSLTPEQWKSHRSYSCQVTHEGSTVEKTVAPTECS

SEQ ID NO: 57 - protein, 122 aa, Homo sapiens; identical to SEQ ID NO: 27

SEQ ID NO: 58 - protein, 122 aa, Homo sapiens
QLQLQESGPGLVKPSETLSLTCTVSGGSISSSSYFWGWIRQPPGKGLEWIGSIYYSGITYYNPSLKSRVTISVDTSKNQFSLKLSSVTAADTAVYYCARHDGATAGLFDYWGQGTLVTVSSA

SEQ ID NO: 59 - protein, 5 aa, Homo sapiens
TYAMN

SEQ ID NO: 60 - protein, 19 aa, Homo sapiens
RIRSKYNNYATYYAASVKG

SEQ ID NO: 61 - protein, 14 aa, Homo sapiens
HGNFGNSYVSWFAY

SEQ ID NO: 62 - protein, 14 aa, Homo sapiens
RSSTGAVTTSNYAN

SEQ ID NO: 63 - protein, 7 aa, Homo sapiens
GTNKRAP

SEQ ID NO: 64 - protein, 9 aa, Homo sapiens
ALWYSNLWV

SEQ ID NO: 65 - protein, 448 aa, Homo sapiens
QLQLQESGPGLVKPSETLSLTCTVSGGSISSGSYFWGWIRQPPGKGLEWIGSIYYSGITYYNPSLKSRVTISVDTSKNQFSLKLSSVTAADTAVYYCARHDGAVAGLFDYWGQGTLVTVSSASTKGPSVFPLAPCSRSTSESTAALGCLVKDYFPEPVTVSWNSGALTSGVHTFPAVLQSSGLYSLSSVVTVPSSSLGTKTYTCNVDHKPSNTKVDKRVESKYGPPCPPCPAPEAAGGPSVFLFPPKPKDTLMISRTPEVTCVVVDVSQEDPEVQFNWYVDGVEVHNAKTKPREEQFNSTYRVVSVLTVLHQDWLNGKEYKCKVSNKGLPSSIEKTISKAKGQPREPQVYTLPPSQEEMTKNQVSLTCLVKGFYPSDIAVEWESNGQPENNYKTTPPVLDSDGSFFLYSRLTVDKSRWQEGNVFSCSVMHEALHNHYTQKSLSLSLGK

SEQ ID NO: 66 - protein, 214 aa, Homo sapiens
SYVLTQPPSVSVAPGQTARITCGGNNIGSKSVHWYQQPPGQAPVVVVYDDSDRPSGIPERFSGSNSGNTATLTISRVEAGDEAVYYCQVWDSSSDHVVFGGGTKLTVLGQPKAAPSVTLFPPSSEELQANKATLVCLISDFYPGAVTVAWKADSSPVKAGVETTTPSKQSNNKYAASSYLSLTPEQWKSHRSYSCQVTHEGSTVEKTVAPTECS

SEQ ID NO: 67 - protein, 448 aa, Homo sapiens; identical to SEQ ID NO: 65

SEQ ID NO: 68 - protein, 448 aa, Homo sapiens
QLQLQESGPGLVKPSETLSLTCTVSGGSISSSSYFWGWIRQPPGKGLEWIGSIYYSGITYYNPSLKSRVTISVDTSKNQFSLKLSSVTAADTAVYYCARHDGAVAGLFDYWGQGTLVTVSSASTKGPSVFPLAPCSRSTSESTAALGCLVKDYFPEPVTVSWNSGALTSGVHTFPAVLQSSGLYSLSSVVTVPSSSLGTKTYTCNVDHKPSNTKVDKRVESKYGPPCPPCPAPEAAGGPSVFLFPPKPKDTLMISRTPEVTCVVVDVSQEDPEVQFNWYVDGVEVHNAKTKPREEQFNSTYRVVSVLTVLHQDWLNGKEYKCKVSNKGLPSSIEKTISKAKGQPREPQVYTLPPSQEEMTKNQVSLTCLVKGFYPSDIAVEWESNGQPENNYKTTPPVLDSDGSFFLYSRLTVDKSRWQEGNVFSCSVMHEALHNHYTQKSLSLSLGK

SEQ ID NO: 69 - protein, 448 aa, Homo sapiens
QLQLQESGPGLVKPSETLSLTCTVSGGSISSGSYFWGWIRQPPGKGLEWIGSIYYSGITYYNPSLKSRVTISVDTSKNQFSLKLSSVTAADTAVYYCARHDGATAGLFDYWGQGTLVTVSSASTKGPSVFPLAPCSRSTSESTAALGCLVKDYFPEPVTVSWNSGALTSGVHTFPAVLQSSGLYSLSSVVTVPSSSLGTKTYTCNVDHKPSNTKVDKRVESKYGPPCPPCPAPEAAGGPSVFLFPPKPKDTLMISRTPEVTCVVVDVSQEDPEVQFNWYVDGVEVHNAKTKPREEQFNSTYRVVSVLTVLHQDWLNGKEYKCKVSNKGLPSSIEKTISKAKGQPREPQVYTLPPSQEEMTKNQVSLTCLVKGFYPSDIAVEWESNGQPENNYKTTPPVLDSDGSFFLYSRLTVDKSRWQEGNVFSCSVMHEALHNHYTQKSLSLSLGK

SEQ ID NO: 70 - protein, 448 aa, Homo sapiens
QLQLQESGPGLVKPSETLSLTCTVSGGSISSGSYFWGWIRQPPGKGLEWIGSIYYSGSTYYNPSLKSRVTISVDTSKNQFSLKLSSVTAADTAVYYCARHDGAVAGLFDYWGQGTLVTVSSASTKGPSVFPLAPCSRSTSESTAALGCLVKDYFPEPVTVSWNSGALTSGVHTFPAVLQSSGLYSLSSVVTVPSSSLGTKTYTCNVDHKPSNTKVDKRVESKYGPPCPPCPAPEAAGGPSVFLFPPKPKDTLMISRTPEVTCVVVDVSQEDPEVQFNWYVDGVEVHNAKTKPREEQFNSTYRVVSVLTVLHQDWLNGKEYKCKVSNKGLPSSIEKTISKAKGQPREPQVYTLPPSQEEMTKNQVSLTCLVKGFYPSDIAVEWESNGQPENNYKTTPPVLDSDGSFFLYSRLTVDKSRWQEGNVFSCSVMHEALHNHYTQKSLSLSLGK

SEQ ID NO: 71 - protein, 448 aa, Homo sapiens
QLQLQESGPGLVKPSETLSLTCTVSGGSISSSSYFWGWIRQPPGKGLEWIGSIYYSGITYYNPSLKSRVTISVDTSKNQFSLKLSSVTAADTAVYYCARHDGATAGLFDYWGQGTLVTVSSASTKGPSVFPLAPCSRSTSESTAALGCLVKDYFPEPVTVSWNSGALTSGVHTFPAVLQSSGLYSLSSVVTVPSSSLGTKTYTCNVDHKPSNTKVDKRVESKYGPPCPPCPAPEAAGGPSVFLFPPKPKDTLMISRTPEVTCVVVDVSQEDPEVQFNWYVDGVEVHNAKTKPREEQFNSTYRVVSVLTVLHQDWLNGKEYKCKVSNKGLPSSIEKTISKAKGQPREPQVYTLPPSQEEMTKNQVSLTCLVKGFYPSDIAVEWESNGQPENNYKTTPPVLDSDGSFFLYSRLTVDKSRWQEGNVFSCSVMHEALHNHYTQKSLSLSLGK

SEQ ID NO: 72 - protein, 448 aa, Homo sapiens
QLQLQESGPGLVKPSETLSLTCTVSGGSISSSSYFWGWIRQPPGKGLEWIGSIYYSGRTYYNPSLKSRVTISVDTSKNQFSLKLSSVTAADTAVYYCARHDGATAGLFDYWGQGTLVTVSSASTKGPSVFPLAPCSRSTSESTAALGCLVKDYFPEPVTVSWNSGALTSGVHTFPAVLQSSGLYSLSSVVTVPSSSLGTKTYTCNVDHKPSNTKVDKRVESKYGPPCPPCPAPEAAGGPSVFLFPPKPKDTLMISRTPEVTCVVVDVSQEDPEVQFNWYVDGVEVHNAKTKPREEQFNSTYRVVSVLTVLHQDWLNGKEYKCKVSNKGLPSSIEKTISKAKGQPREPQVYTLPPSQEEMTKNQVSLTCLVKGFYPSDIAVEWESNGQPENNYKTTPPVLDSDGSFFLYSRLTVDKSRWQEGNVFSCSVMHEALHNHYTQKSLSLSLGK

SEQ ID NO: 73 - protein, 327 aa, synthetic construct
  REGION 1..327: note = Description of Artificial Sequence: Synthetic polypeptide
ASTKGPSVFPLAPCSRSTSESTAALGCLVKDYFPEPVTVSWNSGALTSGVHTFPAVLQSSGLYSLSSVVTVPSSSLGTKTYTCNVDHKPSNTKVDKRVESKYGPPCPPCPAPEAAGGPSVFLFPPKPKDTLMISRTPEVTCVVVDVSQEDPEVQFNWYVDGVEVHNAKTKPREEQFNSTYRVVSVLTVLHQDWLNGKEYKCKVSNKGLPSSIEKTISKAKGQPREPQVYTLPPSQEEMTKNQVSLTCLVKGFYPSDIAVEWESNGQPENNYKTTPPVLDSDGSFFLYSRLTVDKSRWQEGNVFSCSVMHEALHNHYTQKSLSLSLGK

SEQ ID NO: 74 - protein, 330 aa, Homo sapiens
ASTKGPSVFPLAPSSKSTSGGTAALGCLVKDYFPEPVTVSWNSGALTSGVHTFPAVLQSSGLYSLSSVVTVPSSSLGTQTYICNVNHKPSNTKVDKKVEPKSCDKTHTCPPCPAPELLGGPSVFLFPPKPKDTLMISRTPEVTCVVVDVSHEDPEVKFNWYVDGVEVHNAKTKPREEQYNSTYRVVSVLTVLHQDWLNGKEYKCKVSNKALPAPIEKTISKAKGQPREPQVYTLPPSREEMTKNQVSLTCLVKGFYPSDIAVEWESNGQPENNYKTTPPVLDSDGSFFLYSKLTVDKSRWQQGNVFSCSVMHEALHNHYTQKSLSLSPGK

SEQ ID NO: 75 - protein, 230 aa, Homo sapiens
QLQLQESGPGLVKPSETLSLTCTVSGGSISSGSYFWGWIRQPPGKGLEWIGSIYYSGITYYNPSLKSRVTISVDTSKNQFSLKLSSVTAADTAVYYCARHDGAVAGLFDYWGQGTLVTVSSASTKGPSVFPLAPSSKSTSGGTAALGCLVKDYFPEPVTVSWNSGALTSGVHTFPAVLQSSGLYSLSSVVTVPSSSLGTQTYICNVNHKPSNTKVDKKVEPKSCHHHHHH

SEQ ID NO: 76 - protein, 214 aa, Homo sapiens
SYVLTQPPSVSVAPGQTARITCGGNNIGSKSVHWYQQPPGQAPVVVVYDDSDRPSGIPERFSGSNSGNTATLTISRVEAGDEAVYYCQVWDSSSDHVVFGGGTKLTVLGQPKAAPSVTLFPPSSEELQANKATLVCLISDFYPGAVTVAWKGDSSPVKAGVETTTPSKQSNNKYAASSYLSLTPEQWKSHRSYSCQVTHEGSTVEKTVAPTECS

SEQ ID NO: 77 - protein, 5 aa, Homo sapiens
GAVAG